European Patent Application EP 4 621 068 A1, published September 24, 2025. Title: DETECTION OF TARGET NUCLEIC ACID BY QUENCHING-PTO CLEAVAGE AND EXTENSION ASSAY. Applicant: SEEGENE, INC. The sequence listing filed with the application follows.

SEQUENCE LISTING (8 sequences)

SEQ ID NO: 1 - DNA, 22 bp, synthetic construct
  source 1..22: mol_type = other DNA
actgatgtagctgttgctattc

SEQ ID NO: 2 - DNA, 21 bp, synthetic construct
  source 1..21: mol_type = other DNA
aattgttgggtttgtagaagc

SEQ ID NO: 3 - DNA, 43 bp, synthetic construct
  source 1..43: mol_type = other DNA
gccattactgacgagggcatgctccagatattctagaaactgt

SEQ ID NO: 4 - DNA, 36 bp, synthetic construct
  source 1..36: mol_type = other DNA
acgtcgatctatcaatgaatactcgtcagtaatggc

SEQ ID NO: 5 - DNA, 25 bp, synthetic construct
  source 1..25: mol_type = other DNA
gagttttaaaatgggaaattctggt

SEQ ID NO: 6 - DNA, 25 bp, synthetic construct
  source 1..25: mol_type = other DNA
ccaattgtaatagaagcattggttg

SEQ ID NO: 7 - DNA, 39 bp, synthetic construct
  source 1..39: mol_type = other DNA
gattacgcgaccgcatcagaagctgtcattttggctgcg

SEQ ID NO: 8 - DNA, 39 bp, synthetic construct
  source 1..39: mol_type = other DNA
tttttttttttttttttttttatgtgcggtcgcgtaatc